European Patent Specification EP 4 244 361 B1, published February 21, 2024. Title: Fluorescent Fusion Based Heterologous Peptide Production. Applicant: Stellenbosch University. The sequence listing filed with the application follows.

SEQUENCE LISTING (111 sequences)

SEQ ID NO: 1 - protein, 4 aa, Artificial Sequence
  WelQut Cleavage site amino acid sequence
WELQ

SEQ ID NO: 2 - DNA, 12 bp, Artificial sequence
  WelQut Cleavage site nucleotide sequence
tgggaactgcag

SEQ ID NO: 3 - protein, 4 aa, Artificial sequence
  Thrombin/trypsin cleavage site amino acid sequence
LVPR

SEQ ID NO: 4 - DNA, 12 bp, Artificial sequence
  Thrombin/trypsin cleavage site nucleotide sequence
ctagtaccacgc

SEQ ID NO: 5 - protein, 4 aa, Artificial sequence
  nisP/trypsin cleavage site amino acid sequence
ASPR

SEQ ID NO: 6 - DNA, 12 bp, Artificial sequence
  nisP/trypsin cleavage site nucleotide sequence
gcgagcccgcgc

SEQ ID NO: 7 - protein, 7 aa, Artificial sequence
  TEV cleavage site amino acid sequence
ENLYFQG

SEQ ID NO: 8 - DNA, 21 bp, Artificial sequence
  TEV cleavage site nucleotide sequence
gaaaacttgtattttcaaggc

SEQ ID NO: 9 - protein, 4 aa, Artificial sequence
  Factor Xa cleavage site amino acid sequence
IEGR

SEQ ID NO: 10 - DNA, 12 bp, Artificial sequence
  Factor Xa cleavage site nucleotide sequence
attgaaggtcgt

SEQ ID NO: 11 - protein, 240 aa, Artificial sequence
  green fluorescent protein amino acid sequence
MSKGEELFTGVVPILVELDGDVNGYKFSVSGEGEGDATYGKLTLKFICTTGKLPVPWPTLVTTLTYGVQCFSRYPDHMKRHDFFKSAMPEGYVQERTIFFKDDGNYKTRAEVKFEGDTLVNRIELKGIDFKEDGNILGHKLEYNYNSHNVYIMADKQKNGIKANFKTRHNIEDGGVQLADHYQQNTPIGDDPVLLPDNHYLSTQSALSKDPNEKRDHMVLLEFVTAAGITHGMDELYKTG

SEQ ID NO: 12 - DNA, 720 bp, Artificial sequence
  green fluorescent protein nucleotide sequence
atgagtaaaggagaagaacttttcactggagttgtcccaattcttgttgaattagatggtgatgttaatgggtacaaattttctgtcagtggagagggtgaaggtgatgcaacatacggaaaacttacccttaaatttatttgcactactggaaaactacctgttccatggccaacacttgtcactactctcacttatggtgttcaatgcttttcaagatatccagatcatatgaagcggcacgacttcttcaagagcgccatgcctgagggatacgtgcaggagaggaccatcttcttcaaggacgacgggaactacaagacacgtgctgaagtcaagtttgagggagacaccctcgtcaacaggatcgagcttaagggaatcgatttcaaggaggacggaaacatcctcggccacaagttggaatacaactacaactcccacaacgtatacatcatggccgacaagcaaaagaacggcatcaaagccaacttcaagacccgccacaacatcgaagacggcggcgtgcaactcgctgatcattatcaacaaaatactccaattggcgatgaccctgtccttttaccagacaaccattacctgtccacacaatctgccctttcgaaagatcccaacgaaaagagagaccacatggtccttcttgagtttgtaacggctgctgggattacacatggcatggatgaactatacaaaaccggt

SEQ ID NO: 13 - protein, 227 aa, Artificial sequence
  mCherry amino acid sequence
VAIIKEFMRFKVHMEGSVNGHEFEIEGEGEGRPYEGTQTAKLKVTKGGPLPFAWDILSPQFMYGSKAYVKHPADIPDYLKLSFPEGFKWERVMNFEDGGVVTVTQDSSLQDGEFIYKVKLRGTNFPSDGPVMQKKTMGWEASSERMYPEDGALKGEIKQRLKLKDGGHYDAEVKTTYKAKKPVQLPGAYNVNIKLDITSHNEDYTIVEQYERAEGRHSTGGMDELYK

SEQ ID NO: 14 - DNA, 681 bp, Artificial sequence
  mCherry nucleotide sequence
gtggcaatcatcaaagaatttatgcggtttaaagtacatatggaaggtagtgtgaatggtcatgaatttgaaattgaaggtgaaggagaaggtagaccatatgaaggaacgcaaaccgcgaaattgaaagttactaaaggtggaccattaccttttgcatgggatatcttatctccacaatttatgtatggatcaaaagcatatgtaaaacatccagcagatatccctgattatttaaaattaagttttcctgaaggttttaaatgggaacgggttatgaattttgaagatggtggagttgtaactgtaacacaagatagttctttacaagatggagaatttatctataaagtcaaattgcgtggaacgaattttccatctgatggtcctgtgatgcaaaagaaaactatgggttgggaagctagtagtgaacgtatgtatccagaagatggagcattaaaaggtgaaatcaaacaaagattaaaattgaaagatggtggacattatgatgcggaagttaaaactacatataaagccaaaaaaccagtccaattacctggtgcttataatgtgaatatcaaattggatatcacgagtcataatgaagattataccattgtcgaacaatatgaaagagcggaaggaagacattctacaggtggtatggatgaattatataaa

SEQ ID NO: 15 - protein, 161 aa, Artificial sequence
  GpR lytic protein amino acid sequence
MADLVEINNQRKAFLDMLAWSEGTDNGRQKTRNHGYDVIVGGELFTDYSDHPRKLVTLNPKLKSTGAGRYQLLSRWWDAYRKQLGLKDFSPKSQDAVALQQIKERGALPMIDRGDIRQAIDRCSNIWASLPGAGYGQFEHKADSLIAKFKEAGGTVREIDV

SEQ ID NO: 16 - DNA, 483 bp, Artificial sequence
  GpR lytic protein nucleotide sequence
atggcagatctggtagaaatcaataatcaacgtaaggcgttcctcgatatgctggcgtggtcggagggaactgataacggacgtcagaaaaccagaaatcatggttatgacgtcattgtaggcggagagctatttactgattactccgatcaccctcgcaaacttgtcacgctaaacccaaaactcaaatcaacaggcgccggacgctaccagcttctttcccgttggtgggatgcctaccgcaagcagcttggcctgaaagacttctctccgaaaagtcaggacgctgtggcattgcagcagattaaggagcgtggcgctttacctatgattgatcgtggtgatatccgtcaggcaatcgaccgttgcagcaatatctgggcttcactgccgggcgctggttatggtcagttcgagcataaggctgacagcctgattgcaaaattcaaagaagcgggcggaacggtcagagagattgatgta

SEQ ID NO: 17 - protein, 167 aa, Artificial sequence
  GpE lytic protein amino acid sequence
MADLNIFEMLRIDERLRLKIYKDTEGYYTIGIGHLLTKSPSLNAAKSELDKAIGRNCNGVITKDEAEKLFNQDVDAAVRGILRNAKLKPVYDSLDAVRRCALINMVFQMGETGVAGFTNSLRMLQQKRWDEAAVNLAKSIWYNQTPNRAKRVITTFRTGTWDAYKNL

SEQ ID NO: 18 - DNA, 501 bp, Artificial sequence
  GpE lytic protein nucleotide sequence
atggcagatctgaatatttttgaaatgctgcgtatagatgaaggtcttagacttaaaatctataaagacacagaaggctattacactattggcatcggtcatttgcttacaaaaagtccatcacttagtgttgctaaatctgaattagataaagctattggacgtaattgcaatggtgtaattacaaaagatgaggctgaaaaactctttaatcaggatgttgatgctgctgttcgcggaattctgagaaatgctaaattaaaaccggtttatgattctcttgatgcggttcgtcgttgtgcattgattaatatggtcttccaaatgggagaaaccggtgtggcaggatttactaactctttacgtatgcttcaacaaaaacgctgggatgaagcagcagttaacttagctaaaagtagatggtataatcaaacacctaatcgcgcaaaacgagtcattacaacgtttagaactggcacttgggacgcatataaaaatctg

SEQ ID NO: 19 - RNA, 25 nt, Artificial sequence
  RNA thermometer 1
uaguucuccuucagaaggagauaua

SEQ ID NO: 20 - RNA, 130 nt, Artificial sequence
  RNA thermometer 2
uguaaaaaacaucauuuagcgugacuuucuuucaacagcuaacaauuguuguuacugccuaauguuuuuaggguauuuuaaaaaagggcgauaaaaaacgauugggggaugagacaugaacgcucaagca

SEQ ID NO: 21 - RNA, 89 nt, Artificial sequence
  RNA thermometer 3
ggccacuuuagucugugguuacuguauuagguauuguuauaacaaucuggaugguuuuuaugaauaagacauuacuggucucuucuuua

SEQ ID NO: 22 - RNA, 112 nt, Artificial sequence
  RNA thermometer 4
uguguuuuuuguaaguucuauuaaauacaucaguuuacagcaaugaauucaccauugugcaucgucaauaaaaggaguguuuaugaaaaaucaauggcaacaucaauauuuu

SEQ ID NO: 23 - RNA, 46 nt, Artificial sequence
  RNA thermometer 5
acagcaauuuugcguuaccuguuaaucgagauugaaacacaugaaa

SEQ ID NO: 24 - RNA, 240 nt, Artificial sequence
  RNA thermometer 6
ggcgccacgguuugacguacagaccauuaaagcaguguaguaaggcaagucccuucaagaguuaucguugauaccccucguagugcacauuccuuuaacgcuucaaaaucuguaaagcacgccauaucgccgaaaggcacacuuaauuauuaaagguaauacacuauguccgguaaaaugacugguaucguaaaaugguucaacgcugacaaaggcuucggcuucaucacuccugacgau

SEQ ID NO: 25 - RNA, 46 nt, Artificial sequence
  RNA thermometer 7
acagcaauuuugcguuaucuguuaaucgagacugaaauacaugaaa

SEQ ID NO: 26 - RNA, 50 nt, Artificial sequence
  RNA thermometer 8
auucaaggguaaucaauuccuuccacacaucaggaguuaacauuaugucu

SEQ ID NO: 27 - RNA, 110 nt, Artificial sequence
  RNA thermometer 9
ggccuaauuauagcacuuaaucgaaauaaauuuaugaguacguagaguauaauuaguauucuucuuuccaacuuccuuauacuuauauacuuauagauucuaaaaucaug

SEQ ID NO: 28 - protein, 301 aa, Artificial sequence
  GFPNisin (ASPR) amino acid sequence
MSKGEELFTGVVPILVELDGDVNGYKFSVSGEGEGDATYGKLTLKFICTTGKLPVPWPTLVTTLTYGVQCFSRYPDHMKRHDFFKSAMPEGYVQERTIFFKDDGNYKTRAEVKFEGDTLVNRIELKGIDFKEDGNILGHKLEYNYNSHNVYIMADKQKNGIKANFKTRHNIEDGGVQLADHYQQNTPIGDDPVLLPDNHYLSTQSALSKDPNEKRDHMVLLEFVTAAGITHGMDELYKTGWELQMSTKDFNLDLVSVSKKDSGASPRITSISLCTPGCKTGALMGCNMKTATCHCSIHVSK

SEQ ID NO: 29 - DNA, 903 bp, Artificial sequence
  GFPNisin (ASPR) nucleotide sequence
atgagtaaaggagaagaacttttcactggagttgtcccaattcttgttgaattagatggtgatgttaatgggtacaaattttctgtcagtggagagggtgaaggtgatgcaacatacggaaaacttacccttaaatttatttgcactactggaaaactacctgttccatggccaacacttgtcactactctcacttatggtgttcaatgcttttcaagatatccagatcatatgaagcggcacgacttcttcaagagcgccatgcctgagggatacgtgcaggagaggaccatcttcttcaaggacgacgggaactacaagacacgtgctgaagtcaagtttgagggagacaccctcgtcaacaggatcgagcttaagggaatcgatttcaaggaggacggaaacatcctcggccacaagttggaatacaactacaactcccacaacgtatacatcatggccgacaagcaaaagaacggcatcaaagccaacttcaagacccgccacaacatcgaagacggcggcgtgcaactcgctgatcattatcaacaaaatactccaattggcgatgaccctgtccttttaccagacaaccattacctgtccacacaatctgccctttcgaaagatcccaacgaaaagagagaccacatggtccttcttgagtttgtaacggctgctgggattacacatggcatggatgaactatacaaaaccggttgggaactgcagatgagtacaaaagattttaacttggatttggtatctgtttcgaagaaagattcaggtgcatcaccacgcattacaagtatttcgctatgtacacccggttgtaaaacaggagctctgatgggttgtaacatgaaaacagcaacttgtcattgtagtattcacgtaagcaaa

SEQ ID NO: 30 - protein, 315 aa, Artificial sequence
  GFPNisin (AVPR) amino acid sequence
MGSSHHHHHHSQDPMSKGEELFTGVVPILVELDGDVNGYKFSVSGEGEGDATYGKLTLKFICTTGKLPVPWPTLVTTLTYGVQCFSRYPDHMKRHDFFKSAMPEGYVQERTIFFKDDGNYKTRAEVKFEGDTLVNRIELKGIDFKEDGNILGHKLEYNYNSHNVYIMADKQKNGIKANFKTRHNIEDGGVQLADHYQQNTPIGDDPVLLPDNHYLSTQSALSKDPNEKRDHMVLLEFVTAAGITHGMDELYKTGWELQMSTKDFNLDLVSVSKKDSGAVPRITSISLCTPGCKTGALMGCNMKTATCHCSIHVSK

SEQ ID NO: 31 - DNA, 945 bp, Artificial sequence
  GFPNisin (AVPR) nucleotide sequence
atgggcagcagccatcaccatcatcaccacagccaggatccgatgagtaaaggagaagaacttttcactggagttgtcccaattcttgttgaattagatggtgatgttaatgggtacaaattttctgtcagtggagagggtgaaggtgatgcaacatacggaaaacttacccttaaatttatttgcactactggaaaactacctgttccatggccaacacttgtcactactctcacttatggtgttcaatgcttttcaagatatccagatcatatgaagcggcacgacttcttcaagagcgccatgcctgagggatacgtgcaggagaggaccatcttcttcaaggacgacgggaactacaagacacgtgctgaagtcaagtttgagggagacaccctcgtcaacaggatcgagcttaagggaatcgatttcaaggaggacggaaacatcctcggccacaagttggaatacaactacaactcccacaacgtatacatcatggccgacaagcaaaagaacggcatcaaagccaacttcaagacccgccacaacatcgaagacggcggcgtgcaactcgctgatcattatcaacaaaatactccaattggcgatgaccctgtccttttaccagacaaccattacctgtccacacaatctgccctttcgaaagatcccaacgaaaagagagaccacatggtccttcttgagtttgtaacggctgctgggattacacatggcatggatgaactatacaaaaccggttgggaactgcagatgagtacaaaagattttaacttggatttggtatctgtttcgaagaaagattcaggtgcagtaccacgcattacaagtatttcgctatgtacacccggttgtaaaacaggagctctgatgggttgtaacatgaaaacagcaacttgtcattgtagtattcacgtaagcaaa

SEQ ID NO: 32 - protein, 301 aa, Artificial sequence
  GFPMunX amino acid sequence
MGSSHHHHHHSQDPMSKGEELFTGVVPILVELDGDVNGYKFSVSGEGEGDATYGKLTLKFICTTGKLPVPWPTLVTTLTYGVQCFSRYPDHMKRHDFFKSAMPEGYVQERTIFFKDDGNYKTRAEVKFEGDTLVNRIELKGIDFKEDGNILGHKLEYNYNSHNVYIMADKQKNGIKANFKTRHNIEDGGVQLADHYQQNTPIGDDPVLLPDNHYLSTQSALSKDPNEKRDHMVLLEFVTAAGITHGMDELYKTGWELQKYYGNGVSCNKKGCSVDWGKAIGIIGNNSAANLATGGAAGWKS

SEQ ID NO: 33 - DNA, 903 bp, Artificial sequence
  GFPMunX nucleotide sequence
atgggcagcagccatcaccatcatcaccacagccaggatccgatgagtaaaggagaagaacttttcactggagttgtcccaattcttgttgaattagatggtgatgttaatgggtacaaattttctgtcagtggagagggtgaaggtgatgcaacatacggaaaacttacccttaaatttatttgcactactggaaaactacctgttccatggccaacacttgtcactactctcacttatggtgttcaatgcttttcaagatatccagatcatatgaagcggcacgacttcttcaagagcgccatgcctgagggatacgtgcaggagaggaccatcttcttcaaggacgacgggaactacaagacacgtgctgaagtcaagtttgagggagacaccctcgtcaacaggatcgagcttaagggaatcgatttcaaggaggacggaaacatcctcggccacaagttggaatacaactacaactcccacaacgtatacatcatggccgacaagcaaaagaacggcatcaaagccaacttcaagacccgccacaacatcgaagacggcggcgtgcaactcgctgatcattatcaacaaaatactccaattggcgatgaccctgtccttttaccagacaaccattacctgtccacacaatctgccctttcgaaagatcccaacgaaaagagagaccacatggtccttcttgagtttgtaacggctgctgggattacacatggcatggatgaactatacaaaaccggttgggaactgcagaaatactacggtaatggagtctcatgtaataaaaaagggtgcagtgttgattggggaaaagctattggcattattggaaataattctgctgcgaatttagctactggtggagcagctggttggaaaagt

SEQ ID NO: 34 - protein, 295 aa, Artificial sequence
  GFPPlantX amino acid sequence
MGSSHHHHHHSQDPMSKGEELFTGVVPILVELDGDVNGYKFSVSGEGEGDATYGKLTLKFICTTGKLPVPWPTLVTTLTYGVQCFSRYPDHMKRHDFFKSAMPEGYVQERTIFFKDDGNYKTRAEVKFEGDTLVNRIELKGIDFKEDGNILGHKLEYNYNSHNVYIMADKQKNGIKANFKTRHNIEDGGVQLADHYQQNTPIGDDPVLLPDNHYLSTQSALSKDPNEKRDHMVLLEFVTAAGITHGMDELYKTGWELQKYYGNGVTCGKHSCSVNWGQAFSCSVSHLANFGHGKC

SEQ ID NO: 35 - DNA, 885 bp, Artificial sequence
  GFPPlantX nucleotide sequence
atgggcagcagccatcaccatcatcaccacagccaggatccgatgagtaaaggagaagaacttttcactggagttgtcccaattcttgttgaattagatggtgatgttaatgggtacaaattttctgtcagtggagagggtgaaggtgatgcaacatacggaaaacttacccttaaatttatttgcactactggaaaactacctgttccatggccaacacttgtcactactctcacttatggtgttcaatgcttttcaagatatccagatcatatgaagcggcacgacttcttcaagagcgccatgcctgagggatacgtgcaggagaggaccatcttcttcaaggacgacgggaactacaagacacgtgctgaagtcaagtttgagggagacaccctcgtcaacaggatcgagcttaagggaatcgatttcaaggaggacggaaacatcctcggccacaagttggaatacaactacaactcccacaacgtatacatcatggccgacaagcaaaagaacggcatcaaagccaacttcaagacccgccacaacatcgaagacggcggcgtgcaactcgctgatcattatcaacaaaatactccaattggcgatgaccctgtccttttaccagacaaccattacctgtccacacaatctgccctttcgaaagatcccaacgaaaagagagaccacatggtccttcttgagtttgtaacggctgctgggattacacatggcatggatgaactatacaaaaccggttgggaactgcagaaatactatggtaatggggttacttgtggtaaacattcctgctctgttaactggggccaagcattttcttgtagtgtgtcacatttagctaacttcggtcatggaaagtgc

SEQ ID NO: 36 - DNA, 3829 bp, Artificial sequence
  pTAP (RNA thermometer backbone vector) nucleotide sequence
ggggaattgtgagcggataacaattcccctgtagaaataattttgtttaactttaataaggagatataccatgggcagcagccatcaccatcatcaccacagccaggatccgaattcgagctcggcgcgcctgcaggtcgacaagcttgcggccgcataatgcttaagtcgaacagaaagtaatcgtattgtacacggccgcataatcgaaattaatacgactcactataggggaattgtgagcggataacaattccccatcttagtatattagttctccttcagaaggagatatacatatggcagatctcaattggatatcggccggccacgcgatcgctgacgtcggtaccctcgagtctggtaaagaaaccgctgctgcgaaatttgaacgccagcacatggactcgtctactagcgcagcttaattaacctaggctgctgccaccgctgagcaataactagcataaccccttggggcctctaaacgggtcttgaggggttttttgctgaaacctcaggcatttgagaagcacacggtcacactgcttccggtagtcaataaaccggtaaaccagcaatagacataagcggctatttaacgaccctgccctgaaccgacgacaagctgacgaccgggtctccgcaagtggcacttttcggggaaatgtgcgcggaacccctatttgtttatttttctaaatacattcaaatatgtatccgctcatgaattaattcttagaaaaactcatcgagcatcaaatgaaactgcaatttattcatatcaggattatcaataccatatttttgaaaaagccgtttctgtaatgaaggagaaaactcaccgaggcagttccataggatggcaagatcctggtatcggtctgcgattccgactcgtccaacatcaatacaacctattaatttcccctcgtcaaaaataaggttatcaagtgagaaatcaccatgagtgacgactgaatccggtgagaatggcaaaagtttatgcatttctttccagacttgttcaacaggccagccattacgctcgtcatcaaaatcactcgcatcaaccaaaccgttattcattcgtgattgcgcctgagcgagacgaaatacgcggtcgctgttaaaaggacaattacaaacaggaatcgaatgcaaccggcgcaggaacactgccagcgcatcaacaatattttcacctgaatcaggatattcttctaatacctggaatgctgttttcccggggatcgcagtggtgagtaaccatgcatcatcaggagtacggataaaatgcttgatggtcggaagaggcataaattccgtcagccagtttagtctgaccatctcatctgtaacatcattggcaacgctacctttgccatgtttcagaaacaactctggcgcatcgggcttcccatacaatcgatagattgtcgcacctgattgcccgacattatcgcgagcccatttatacccatataaatcagcatccatgttggaatttaatcgcggcctagagcaagacgtttcccgttgaatatggctcatactcttcctttttcaatattattgaagcatttatcagggttattgtctcatgagcggatacatatttgaatgtatttagaaaaataaacaaataggcatgcagcgctcttccgcttcctcgctcactgactcgctacgctcggtcgttcgactgcggcgagcggtgtcagctcactcaaaagcggtaatacggttatccacagaatcaggggataaagccggaaagaacatgtgagcaaaaagcaaagcaccggaagaagccaacgccgcaggcgtttttccataggctccgcccccctgacgagcatcacaaaaatcgacgctcaagccagaggtggcgaaacccgacaggactataaagataccaggcgtttccccctggaagctccctcgtgcgctctcctgttccgaccctgccgcttaccggatacctgtccgcctttctcccttcgggaagcgtggcgctttctcatagctcacgctgttggtatctcagttcggtgtaggtcgttcgctccaagctgggctgtgtgcacgaaccccccgttcagcccgaccgctgcgccttatccggtaactatcgtcttgagtccaacccggtaagacacgacttatcgccactggcagcagccattggtaactgatttagaggactttgtcttgaagttatgcacctgttaaggctaaactgaaagaacagattttggtgagtgcggtcctccaacccacttaccttggttcaaagagttggtagctcagcgaaccttgagaaaaccaccgttggtagcggtggtttttctttatttatgagatgatgaatcaatcggtctatcaagtcaacgaacagctattccgttactctagatttcagtgcaatttatctcttcaaatgtagcacctgaagtcagccccatacgatataagttgtaattctcatgttagtcatgccccgcgcccaccggaaggagctgactgggttgaaggctctcaagggcatcggtcgagatcccggtgcctaatgagtgagctaacttacattaattgcgttgcgctcactgcccgctttccagtcgggaaacctgtcgtgccagctgcattaatgaatcggccaacgcgcggggagaggcggtttgcgtattgggcgccagggtggtttttcttttcaccagtgagacgggcaacagctgattgcccttcaccgcctggccctgagagagttgcagcaagcggtccacgctggtttgccccagcaggcgaaaatcctgtttgatggtggttaacggcgggatataacatgagctgtcttcggtatcgtcgtatcccactaccgagatgtccgcaccaacgcgcagcccggactcggtaatggcgcgcattgcgcccagcgccatctgatcgttggcaaccagcatcgcagtgggaacgatgccctcattcagcatttgcatggtttgttgaaaaccggacatggcactccagtcgccttcccgttccgctatcggctgaatttgattgcgagtgagatatttatgccagccagccagacgcagacgcgccgagacagaacttaatgggcccgctaacagcgcgatttgctggtgacccaatgcgaccagatgctccacgcccagtcgcgtaccgtcttcatgggagaaaataatactgttgatgggtgtctggtcagagacatcaagaaataacgccggaacattagtgcaggcagcttccacagcaatggcatcctggtcatccagcggatagttaatgatcagcccactgacgcgttgcgcgagaagattgtgcaccgccgctttacaggcttcgacgccgcttcgttctaccatcgacaccaccacgctggcacccagttgatcggcgcgagatttaatcgccgcgacaatttgcgacggcgcgtgcagggccagactggaggtggcaacgccaatcagcaacgactgtttgcccgccagttgttgtgccacgcggttgggaatgtaattcagctccgccatcgccgcttccactttttcccgcgttttcgcagaaacgtggctggcctggttcaccacgcgggaaacggtctgataagagacaccggcatactctgcgacatcgtataacgttactggtttcacattcaccaccctgaattgactctcttccgggcgctatcatgccataccgcgaaaggttttgcgccattcgatggtgtccgggatctcgacgctctcccttatgcgactcctgcattaggaaattaatacgactcactata

SEQ ID NO: 37 - protein, 761 aa, Artificial sequence
  GFPLLO amino acid sequence
MGSSHHHHHHSQDPMSKGEELFTGVVPILVELDGDVNGYKFSVSGEGEGDATYGKLTLKFICTTGKLPVPWPTLVTTLTYGVQCFSRYPDHMKRHDFFKSAMPEGYVQERTIFFKDDGNYKTRAEVKFEGDTLVNRIELKGIDFKEDGNILGHKLEYNYNSHNVYIMADKQKNGIKANFKTRHNIEDGGVQLADHYQQNTPIGDDPVLLPDNHYLSTQSALSKDPNEKRDHMVLLEFVTAAGITHGMDELYKTGWELQASAFNKENSISSMAPPASPPASPKTPIEKKHADEIDKYIQGLDYNKNNVLVYHGDAVTNVPPRKGYKDGNEYIVVEKKKKSINQNNADIQVVNAISSLTYPGALVKANSELVENQPDVLPVKRDSLTLSIDLPGMTNQDNKIVVKNATKSNVNNAVNTLVERWNEKYAQAYPNVSAKIDYDDEMAYSESQLIAKFGTAFKAVNNSLNVNFGAISEGKMQEEVISFKQIYYNVNVNEPTRPSRFFGKAVTKEQLQALGVNAENPPAYISSVAYGRQVYLKLSTNSHSTKVKAAFDAAVSGKSVSGDVELTNIIKNSSFKAVIYGGSAKDEVQIIDGNLGDLRDILKKGATFNRETPGVPIAYTTNFLKDNELAVIKNNSEYIETTSKAYTDGKINIDHSGGYVAQFNISWDEVNYDPEGNEIVQHKNWSENNKSKLAHFTSSIYLPGNARNINVYAKECTGLAWEWWRTVIDDRNLPLVKNRNISIWGTTLYPKYSNKVDNPIE

SEQ ID NO: 38 - DNA, 2283 bp, Artificial sequence
  GFPLLO nucleotide sequence
atgggcagcagccatcaccatcatcaccacagccaggatccgatgagtaaaggagaagaacttttcactggagttgtcccaattcttgttgaattagatggtgatgttaatgggtacaaattttctgtcagtggagagggtgaaggtgatgcaacatacggaaaacttacccttaaatttatttgcactactggaaaactacctgttccatggccaacacttgtcactactctcacttatggtgttcaatgcttttcaagatatccagatcatatgaagcggcacgacttcttcaagagcgccatgcctgagggatacgtgcaggagaggaccatcttcttcaaggacgacgggaactacaagacacgtgctgaagtcaagtttgagggagacaccctcgtcaacaggatcgagcttaagggaatcgatttcaaggaggacggaaacatcctcggccacaagttggaatacaactacaactcccacaacgtatacatcatggccgacaagcaaaagaacggcatcaaagccaacttcaagacccgccacaacatcgaagacggcggcgtgcaactcgctgatcattatcaacaaaatactccaattggcgatgaccctgtccttttaccagacaaccattacctgtccacacaatctgccctttcgaaagatcccaacgaaaagagagaccacatggtccttcttgagtttgtaacggctgctgggattacacatggcatggatgaactatacaaaaccggttgggaactgcaggcatctgcattcaataaagaaaattcaatttcatccatggcaccaccagcatctccgcctgcaagtcctaagacgccaatcgaaaagaaacacgcggatgaaatcgataagtatatacaaggattggattacaataaaaacaatgtattagtataccacggagatgcagtgacaaatgtgccgccaagaaaaggttacaaagatggaaatgaatatattgttgtggagaaaaagaagaaatccatcaatcaaaataatgcagacattcaagttgtgaatgcaatttcgagcctaacctatccaggtgctctcgtaaaagcgaattcggaattagtagaaaatcaaccagatgttctccctgtaaaacgtgattcattaacactcagcattgatttgccaggtatgactaatcaagacaataaaatcgttgtaaaaaatgccactaaatcaaacgttaacaacgcagtaaatacattagtggaaagatggaatgaaaaatatgctcaagcttatccaaatgtaagtgcaaaaattgattatgatgacgaaatggcttacagtgaatcacaattaattgcgaaatttggtacagcatttaaagctgtaaataatagcttgaatgtaaacttcggcgcaatcagtgaagggaaaatgcaagaagaagtcattagttttaaacaaatttactataacgtgaatgttaatgaacctacaagaccttccagatttttcggcaaagctgttactaaagagcagttgcaagcgcttggagtgaatgcagaaaatcctcctgcatatatctcaagtgtggcgtatggccgtcaagtttatttgaaattatcaactaattcccatagtactaaagtaaaagctgcttttgatgctgccgtaagcggaaaatctgtctcaggtgatgtagaactaacaaatatcatcaaaaattcttccttcaaagccgtaatttacggaggttccgcaaaagatgaagttcaaatcatcgacggcaacctcggagacttacgcgatattttgaaaaaaggcgctacttttaatcgagaaacaccaggagttcccattgcttatacaacaaacttcctaaaagacaatgaattagctgttattaaaaacaactcagaatatattgaaacaacttcaaaagcttatacagatggaaaaattaacatcgatcactctggaggatacgttgctcaattcaacatttcttgggatgaagtaaattatgatcctgaaggtaacgaaattgttcaacataaaaactggagcgaaaacaataaaagcaagctagctcatttcacatcgtccatctatttgccaggtaacgcgagaaatattaatgtttacgctaaagaatgcactggtttagcttgggaatggtggagaacggtaattgatgaccggaacttaccacttgtgaaaaatagaaatatctccatctggggcaccacgctttatccgaaatatagtaataaagtagataatccaatcgaa

SEQ ID NO: 39 - protein, 1065 aa, Artificial sequence
  GFPActA amino acid sequence
MGSSHHHHHHSQDPMSKGEELFTGVVPILVELDGDVNGYKFSVSGEGEGDATYGKLTLKFICTTGKLPVPWPTLVTTLTYGVQCFSRYPDHMKRHDFFKSAMPEGYVQERTIFFKDDGNYKTRAEVKFEGDTLVNRIELKGIDFKEDGNILGHKLEYNYNSHNVYIMADKQKNGIKANFKTRHNIEDGGVQLADHYQQNTPIGDDPVLLPDNHYLSTQSALSKDPNEKRDHMVLLEFVTAAGITHGMDELYKTGWELQDSEDSSLNTDEWEEEKTEEQPSEVNTGPRYETAREVSSRDIKELEKSNKVRNTNKADLIAMLKEKAEKGPNINNNNSEQTENAAINEEASGADRPAIQVERRHPGLPSDSAAEIKKRRKAIASSDSELESLTYPDKPTKVNKKKVAKESVADASESDLDSSMQSADESSPQPLKANQQPFFPKVFKKIKDAGKWVRDKIDENPEVKKAIVDKSAGLIDQLLTKKKSEEVNASDFPPPPTDEELRLALPETPMLLGFNAPATSEPSSFEFPPPPTDEELRLALPETPMLLGFNAPATSEPSSFEFPPPPTEDELEIIRETASSLDSSFTRGDLASLRNAINRHSQNFSDFPPIPTEEELNGRGGRPTSEEFSSLNSGDFTDDENSETTEEEIDRLADLRDRGTGKHSRNAGFLPLNPFASSPVPSLSPKVSKISAPALISDITKKTPFKNPSQPLNVFNKKTTTKTVTKKPTPVKTAPKLAELPATKPQETVLRENKTPFIEKQAETNKQSINMPSLPVIQKEATESDKEEMKPQTEEKMVEESESANNANGKNRSAGIEEGKLIAKSAEDEKAKEEPGNHTTAVPRAAASPILGYWKIKGLVQPTRLLLEYLEEKYEEHLYERDEGDKWRNKKFELGLEFPNLPYYIDGDVKLTQSMAIIRYIADKHNMLGGCPKERAEISMLEGAVLDIRYGVSRIAYSKDFETLKVDFLSKLPEMLKMFEDRLCHKTYLNGDHVTHPDFMLYDALDVVLYMDPMCLDAFPKLVCFKKRIEAIPQIDKYLKSSKYIAWPLQGWQATFGGGDHPPKS

SEQ ID NO: 40 - DNA, 3195 bp, Artificial sequence
  GFPActA nucleotide sequence
atgggcagcagccatcaccatcatcaccacagccaggatccgatgagtaaaggagaagaacttttcactggagttgtcccaattcttgttgaattagatggtgatgttaatgggtacaaattttctgtcagtggagagggtgaaggtgatgcaacatacggaaaacttacccttaaatttatttgcactactggaaaactacctgttccatggccaacacttgtcactactctcacttatggtgttcaatgcttttcaagatatccagatcatatgaagcggcacgacttcttcaagagcgccatgcctgagggatacgtgcaggagaggaccatcttcttcaaggacgacgggaactacaagacacgtgctgaagtcaagtttgagggagacaccctcgtcaacaggatcgagcttaagggaatcgatttcaaggaggacggaaacatcctcggccacaagttggaatacaactacaactcccacaacgtatacatcatggccgacaagcaaaagaacggcatcaaagccaacttcaagacccgccacaacatcgaagacggcggcgtgcaactcgctgatcattatcaacaaaatactccaattggcgatgaccctgtccttttaccagacaaccattacctgtccacacaatctgccctttcgaaagatcccaacgaaaagagagaccacatggtccttcttgagtttgtaacggctgctgggattacacatggcatggatgaactatacaaaaccggttgggaactgcaggatagcgaagattctagtctaaacacagatgaatgggaagaagaaaaaacagaagagcaaccaagcgaggtaaatacgggaccaagatacgaaactgcacgtgaagtaagttcacgtgatattaaagaactagaaaaatcgaataaagtgagaaatacgaacaaagcagacctaatagcaatgttgaaagaaaaagcagaaaaaggtccaaatatcaataataacaacagtgaacaaactgagaatgcggctataaatgaagaggcttcaggagccgaccgaccagctatacaagtggagcgtcgtcatccaggattgccatcggatagcgcagcggaaattaaaaaaagaaggaaagccatagcatcatcggatagtgagcttgaaagccttacttatccggataaaccaacaaaagtaaataagaaaaaagtggcgaaagagtcagttgcggatgcttctgaaagtgacttagattctagcatgcagtcagcagatgagtcttcaccacaacctttaaaagcaaaccaacaaccatttttccctaaagtatttaaaaaaataaaagatgcggggaaatgggtacgtgataaaatcgacgaaaatcctgaagtaaagaaagcgattgttgataaaagtgcagggttaattgaccaattattaaccaaaaagaaaagtgaagaggtaaatgcttcggacttcccgccaccacctacggatgaagagttaagacttgctttgccagagacaccaatgcttcttggttttaatgctcctgctacatcagaaccgagctcattcgaatttccaccaccacctacggatgaagagttaagacttgctttgccagagacgccaatgcttcttggttttaatgctcctgctacatcggaaccgagctcgttcgaatttccaccgcctccaacagaagatgaactagaaatcatccgggaaacagcatcctcgctagattctagttttacaagaggggatttagctagtttgagaaatgctattaatcgccatagtcaaaatttctctgatttcccaccaatcccaacagaagaagagttgaacgggagaggcggtagaccaacatctgaagaatttagttcgctgaatagtggtgattttacagatgacgaaaacagcgagacaacagaagaagaaattgatcgcctagctgatttaagagatagaggaacaggaaaacactcaagaaatgcgggttttttaccattaaatccgtttgctagcagcccggttccttcgttaagtccaaaggtatcgaaaataagcgcaccggctctgataagtgacataactaaaaaaacgccatttaagaatccatcacagccattaaatgtgtttaataaaaaaactacaacgaaaacagtgactaaaaaaccaacccctgtaaagaccgcaccaaagctagcagaacttcctgccacaaaaccacaagaaaccgtacttagggaaaataaaacaccctttatagaaaaacaagcagaaacaaacaagcagtcaattaatatgccgagcctaccagtaatccaaaaagaagctacagagagcgataaagaggaaatgaaaccacaaaccgaggaaaaaatggtagaggaaagcgaatcagctaataacgcaaacggaaaaaatcgttctgctggcattgaagaaggaaaactaattgctaaaagtgcagaagacgaaaaagcgaaggaagaaccagggaaccatacgacggcagtaccacgcgcggccgcgtcccctatactaggttattggaaaattaagggccttgtgcaacccactcgacttcttttggaatatcttgaagaaaaatatgaagagcatttgtatgagcgcgatgaaggtgataaatggcgaaacaaaaagtttgaattgggtttggagtttcccaatcttccttattatattgatggtgatgttaaattaacacagtctatggccatcatacgttatatagctgacaagcacaacatgttgggtggttgtccaaaagagcgtgcagagatttcaatgcttgaaggagcggttttggatattagatacggtgtttcgagaattgcatatagtaaagactttgaaactctcaaagttgattttcttagcaagctacctgaaatgctgaaaatgttcgaagatcgtttatgtcataaaacatatttaaatggtgatcatgtaacccatcctgacttcatgttgtatgacgctcttgatgttgttttatacatggacccaatgtgcctggatgcgttcccaaaattagtttgttttaaaaaacgtattgaagctatcccacaaattgataagtacttgaaatccagcaagtatatagcatggcctttgcagggctggcaagccacgtttggtggtggcgaccatcctccaaaatcg

SEQ ID NO: 41 - DNA, 50 bp, Artificial sequence
  GFP_BamHI_F primer sequence
ggatccgatgagtaaaggagaagaacttttcactggagttgtcccaattc

SEQ ID NO: 42 - DNA, 50 bp, Artificial sequence
  GFPWELQ_PstI_R primer sequence
ctgcagttcccaaccggttttgtatagttcatccatgccatgtgtaatcc

SEQ ID NO: 43 - DNA, 38 bp, Artificial sequence
  NisA_BamHI_F primer sequence
ctagatggatccgatgagtacaaaagattttaacttgg

SEQ ID NO: 44 - DNA, 37 bp, Artificial sequence
  NisA_HindIII_R primer
ctagaagcttttatttgcttacgtgaatactacaatg

SEQ ID NO: 45 - DNA, 43 bp, Artificial sequence
  NisB_BglII_F primer
cagccgagatctgatgataaaaagttcatttaaagctcaaccg

SEQ ID NO: 46 - DNA, 42 bp, Artificial sequence
  NisB_XhoI_R primer
ctagctcgagtcatttcatgtattcttccgaaacaaacaacc

SEQ ID NO: 47 - DNA, 45 bp, Artificial sequence
  NisC_BglII_F primer
ctagggaagatctgatgaataaaaaaaatataaaaagaaatgttg

SEQ ID NO: 48 - DNA, 43 bp, Artificial sequence
  NisC_XhoI_R primer
ctagctcgagtcatttcctcttccctcctttcaaaaaatcgtc

SEQ ID NO: 49 - DNA, 24 bp, Artificial sequence
  GFPNisLeader_PstI_F primer
ggaactgcagatgagtacaaaaga

SEQ ID NO: 50 - DNA, 37 bp, Artificial sequence
  NisinLThPep5_F primer
caggtgcagtaccacgcaccgcgggtccggcgatccg

SEQ ID NO: 51 - DNA, 30 bp, Artificial sequence
  Pep5HindIII_R primer
caccaagcttttatttgcagccgtttttac

SEQ ID NO: 52 - DNA, 37 bp, Artificial sequence
  NisinLTh15X_F primer
caggtgcagtaccacgcagcgcgagcatcgtgaagac

SEQ ID NO: 53 - DNA, 31 bp, Artificial sequence
  15XHindIII_R primer
gcgccaagcttttatttcttgccggtaaagt

SEQ ID NO: 54 - DNA, 21 bp, Artificial sequence
  NisLeaderThr_R primer
gcgtggtactgcacctgaatc

SEQ ID NO: 55 - DNA, 25 bp, Artificial sequence
  NisLeaderOri_F primer
gaaagattcaggtgcatcaccacgc

SEQ ID NO: 56 - DNA, 25 bp, Artificial sequence
  NisLeaderOri_R primer
gcgtggtgatgcacctgaatctttc

SEQ ID NO: 57 - DNA, 30 bp, Artificial sequence
  NisLeaderNisThr_F primer
ttcaggtgcagtaccacgcattacaagtat

SEQ ID NO: 58 - DNA, 30 bp, Artificial sequence
  NisLeaderNisThr_R primer
atacttgtaatgcgtggtactgcacctgaa

SEQ ID NO: 59 - DNA, 33 bp, Artificial sequence
  GFP-PlaX_Pst_Fwd primer
taagggatccgtgggaactgcagaaatactatg

SEQ ID NO: 60 - DNA, 41 bp, Artificial sequence
  GFP-PlaX_Hind_Rev primer
tattaagcttagcactttccatgaccgaagttagctaaatg

SEQ ID NO: 61 - DNA, 47 bp, Artificial sequence
  GFP-MunX_Pst_Fwd primer
atcgctgcagaaatactacggtaatggagtctcatgtaataaaaaag

SEQ ID NO: 62 - DNA, 29 bp, Artificial sequence
  GFP-MunX_Hind_Rev primer
acgcaagcttaacttttccaaccagctgc

SEQ ID NO: 63 - DNA, 20 bp, Artificial sequence
  pRSFMCS1_R primer
gattatgcggccgtgtacaa

SEQ ID NO: 64 - DNA, 35 bp, Artificial sequence
  GST_NotI_F primer
gcgcggccgcgtcccctatactaggttattggaaa

SEQ ID NO: 65 - DNA, 35 bp, Artificial sequence
  GST_XhoI_R primer
cagactcgagttacgattttggaggatggtcgcca

SEQ ID NO: 66 - DNA, 30 bp, Artificial sequence
  WLLO_PstI_F primer
gggaactgcaggcatctgcattcaataaag

SEQ ID NO: 67 - DNA, 30 bp, Artificial sequence
  LLO_NotI_R primer
attatgcggccgcttattcgattggattat

SEQ ID NO: 68 - DNA, 37 bp, Artificial sequence
  WActA_PstI_F primer
gggaactgcaggatagcgaagattctagtctaaacac

SEQ ID NO: 69 - DNA, 30 bp, Artificial sequence
  ActA_NotI_R primer
atgcggccgcttacgtcgtatggttccctg

SEQ ID NO: 70 - DNA, 30 bp, Artificial sequence
  GPR-F primer
atggcagatctggtagaaatcaataatcaa

SEQ ID NO: 71 - DNA, 33 bp, Artificial sequence
  GPR-R primer
ataggtacctcatacatcaatctctctgaccgt

SEQ ID NO: 72 - DNA, 30 bp, Artificial sequence
  GPE-F primer
atggcagatctgaatatttttgaaatgctg

SEQ ID NO: 73 - DNA, 30 bp, Artificial sequence
  GPE-R primer
cagactcgagttacagatttttatatgcat

SEQ ID NO: 74 - DNA, 214 bp, Artificial sequence
  Stationary phase promoter 1
ggcgccctggcacaggaacgttatccggacgttcagttccaccagacccgcgagcattaattcttgcctccagggcgcggtagtcgcgccctgtcaatttcccttccttattagccgcttacggaatgttcttaaaacattcacttttgcttatgttttcgctcatatcccgagcggtttcaaaattgtgatctatatttaacaaattaattaa

SEQ ID NO: 75 - DNA, 231 bp, Artificial sequence
  Stationary phase promoter 2
ggcgcctttgtggtgatctacactgatactctgttgcattattcgcctgaaaccacaatattcaggcgttttttcgctatctttgacaaaaaatatcaactttctcgatttgctctcagcccttatatcacgggaaattccggcgatttgctcgcatcaatattcatgccacatttgccatcaggggccgcctcagattctcagtatgttataatagaaaaaattaattaa

SEQ ID NO: 76 - DNA, 197 bp, Artificial sequence
  Stationary phase promoter 3
ggcgccaaaaaatattcagttacaggaaaggtcagggcagggattctacagagttctggataaaatttgtatcgcaatctcattcgctgccggaggcgaaggaaatgtaaattttgttaattcggcgtgaagaattgatcctggacagcattttgctcaaaaaatagccatactatttaattgcaacaattaattaa

SEQ ID NO: 77 - DNA, 328 bp, Artificial sequence
  Promoter / RNA thermometer combination 1
ggcgccaaaaaatattcagttacaggaaaggtcagggcagggattctacagagttctggataaaatttgtatcgcaatctcattcgctgccggaggcgaaggaaatgtaaattttgttaattcggcgtgaagaattgatcctggacagcattttgctcaaaaaatagccatactatttaattgcaacaattaattaaggcctaattatagcacttaatcgaaataaatttatgagtacgtagagtataattagtattcttctttccaacttccttatacttatatacttatagattctaaaatcatgaaacggattctttgcggatcc

SEQ ID NO: 78 - DNA, 261 bp, Artificial sequence
  Promoter / RNA thermometer combination 2
ggcgccaaaaaatattcagttacaggaaaggtcagggcagggattctacagagttctggataaaatttgtatcgcaatctcattcgctgccggaggcgaaggaaatgtaaattttgttaattcggcgtgaagaattgatcctggacagcattttgctcaaaaaatagccatactatttaattgcaacaattaattaaacagcaattttgcgttatctgttaatcgagactgaaatacatgaaaaaaaccacattaggatcc

SEQ ID NO: 79 - DNA, 437 bp, Artificial sequence
  Promoter / RNA thermometer combination 3
ggcgccaaaaaatattcagttacaggaaaggtcagggcagggattctacagagttctggataaaatttgtatcgcaatctcattcgctgccggaggcgaaggaaatgtaaattttgttaattcggcgtgaagaattgatcctggacagcattttgctcaaaaaatagccatactatttaattgcaacaattaattaaacggtttgacgtacagaccattaaagcagtgtagtaaggcaagtcccttcaagagttatcgttgatacccctcgtagtgcacattcctttaacgcttcaaaatctgtaaagcacgccatatcgccgaaaggcacacttaattattaaaggtaatacactatgtccggtaaaatgactggtatcgtaaaatggttcaacgctgacaaaggcttcggcttcatcactcctgacgatggatcc

SEQ ID NO: 80 - DNA, 261 bp, Artificial sequence
  Promoter / RNA thermometer combination 4
ggcgccaaaaaatattcagttacaggaaaggtcagggcagggattctacagagttctggataaaatttgtatcgcaatctcattcgctgccggaggcgaaggaaatgtaaattttgttaattcggcgtgaagaattgatcctggacagcattttgctcaaaaaatagccatactatttaattgcaacaattaattaaacagcaattttgcgttacctgttaatcgagattgaaacacatgaaaaaaaccacattaggatcc

SEQ ID NO: 81 - DNA, 265 bp, Artificial sequence
  Promoter / RNA thermometer combination 5
ggcgccaaaaaatattcagttacaggaaaggtcagggcagggattctacagagttctggataaaatttgtatcgcaatctcattcgctgccggaggcgaaggaaatgtaaattttgttaattcggcgtgaagaattgatcctggacagcattttgctcaaaaaatagccatactatttaattgcaacaattaattaaattcaagggtaatcaattccttccacacatcaggagttaacattatgtctctcattctttacggatcc

SEQ ID NO: 82 - DNA, 292 bp, Artificial sequence
  Promoter / RNA thermometer combination 6
ggcgccaaaaaatattcagttacaggaaaggtcagggcagggattctacagagttctggataaaatttgtatcgcaatctcattcgctgccggaggcgaaggaaatgtaaattttgttaattcggcgtgaagaattgatcctggacagcattttgctcaaaaaatagccatactatttaattgcaacaattaattaaggccactttagtctgtggttactgtattaggtattgttataacaatctggatggtttttatgaataagacattactggtctcttctttaggatcc

SEQ ID NO: 83 - DNA, 315 bp, Artificial sequence
  Promoter / RNA thermometer combination 7
ggcgccaaaaaatattcagttacaggaaaggtcagggcagggattctacagagttctggataaaatttgtatcgcaatctcattcgctgccggaggcgaaggaaatgtaaattttgttaattcggcgtgaagaattgatcctggacagcattttgctcaaaaaatagccatactatttaattgcaacaattaattaatgtgttttttgtaagttctattaaatacatcagtttacagcaatgaattcaccattgtgcatcgtcaataaaaggagtgtttatgaaaaatcaatggcaacatcaatattttggatcc

SEQ ID NO: 84 - DNA, 345 bp, Artificial sequence
  Promoter / RNA thermometer combination 8
ggcgccctggcacaggaacgttatccggacgttcagttccaccagacccgcgagcattaattcttgcctccagggcgcggtagtcgcgccctgtcaatttcccttccttattagccgcttacggaatgttcttaaaacattcacttttgcttatgttttcgctcatatcccgagcggtttcaaaattgtgatctatatttaacaaattaattaaggcctaattatagcacttaatcgaaataaatttatgagtacgtagagtataattagtattcttctttccaacttccttatacttatatacttatagattctaaaatcatgaaacggattctttgcggatcc

SEQ ID NO: 85 - DNA, 295 bp, Artificial sequence
  Promoter / RNA thermometer combination 9
ggcgcctttgtggtgatctacactgatactctgttgcattattcgcctgaaaccacaatattcaggcgttttttcgctatctttgacaaaaaatatcaactttctcgatttgctctcagcccttatatcacgggaaattccggcgatttgctcgcatcaatattcatgccacatttgccatcaggggccgcctcagattctcagtatgttataatagaaaaaattaattaaacagcaattttgcgttatctgttaatcgagactgaaatacatgaaaaaaaccacattaggatcc

SEQ ID NO: 86 - DNA, 471 bp, Artificial sequence
  Promoter / RNA thermometer combination 10
ggcgcctttgtggtgatctacactgatactctgttgcattattcgcctgaaaccacaatattcaggcgttttttcgctatctttgacaaaaaatatcaactttctcgatttgctctcagcccttatatcacgggaaattccggcgatttgctcgcatcaatattcatgccacatttgccatcaggggccgcctcagattctcagtatgttataatagaaaaaattaattaaacggtttgacgtacagaccattaaagcagtgtagtaaggcaagtcccttcaagagttatcgttgatacccctcgtagtgcacattcctttaacgcttcaaaatctgtaaagcacgccatatcgccgaaaggcacacttaattattaaaggtaatacactatgtccggtaaaatgactggtatcgtaaaatggttcaacgctgacaaaggcttcggcttcatcactcctgacgatggatcc

SEQ ID NO: 87 - DNA, 295 bp, Artificial sequence
  Promoter / RNA thermometer combination 11
ggcgcctttgtggtgatctacactgatactctgttgcattattcgcctgaaaccacaatattcaggcgttttttcgctatctttgacaaaaaatatcaactttctcgatttgctctcagcccttatatcacgggaaattccggcgatttgctcgcatcaatattcatgccacatttgccatcaggggccgcctcagattctcagtatgttataatagaaaaaattaattaaacagcaattttgcgttacctgttaatcgagattgaaacacatgaaaaaaaccacattaggatcc

SEQ ID NO: 88 - DNA, 299 bp, Artificial sequence
  Promoter / RNA thermometer combination 12
ggcgcctttgtggtgatctacactgatactctgttgcattattcgcctgaaaccacaatattcaggcgttttttcgctatctttgacaaaaaatatcaactttctcgatttgctctcagcccttatatcacgggaaattccggcgatttgctcgcatcaatattcatgccacatttgccatcaggggccgcctcagattctcagtatgttataatagaaaaaattaattaaattcaagggtaatcaattccttccacacatcaggagttaacattatgtctctcattctttacggatcc

SEQ ID NO: 89 - DNA, 326 bp, Artificial sequence
  Promoter / RNA thermometer combination 13
ggcgcctttgtggtgatctacactgatactctgttgcattattcgcctgaaaccacaatattcaggcgttttttcgctatctttgacaaaaaatatcaactttctcgatttgctctcagcccttatatcacgggaaattccggcgatttgctcgcatcaatattcatgccacatttgccatcaggggccgcctcagattctcagtatgttataatagaaaaaattaattaaggccactttagtctgtggttactgtattaggtattgttataacaatctggatggtttttatgaataagacattactggtctcttctttaggatcc

SEQ ID NO: 90 - DNA, 349 bp, Artificial sequence
  Promoter / RNA thermometer combination 14
ggcgcctttgtggtgatctacactgatactctgttgcattattcgcctgaaaccacaatattcaggcgttttttcgctatctttgacaaaaaatatcaactttctcgatttgctctcagcccttatatcacgggaaattccggcgatttgctcgcatcaatattcatgccacatttgccatcaggggccgcctcagattctcagtatgttataatagaaaaaattaattaatgtgttttttgtaagttctattaaatacatcagtttacagcaatgaattcaccattgtgcatcgtcaataaaaggagtgtttatgaaaaatcaatggcaacatcaatattttggatcc

SEQ ID NO: 91 - DNA, 373 bp, Artificial sequence
  Promoter / RNA thermometer combination 15
ggcgcctttgtggtgatctacactgatactctgttgcattattcgcctgaaaccacaatattcaggcgttttttcgctatctttgacaaaaaatatcaactttctcgatttgctctcagcccttatatcacgggaaattccggcgatttgctcgcatcaatattcatgccacatttgccatcaggggccgcctcagattctcagtatgttataatagaaaaaattaattaatgtaaaaaacatcatttagcgtgactttctttcaacagctaacaattgttgttactgcctaatgtttttagggtattttaaaaaagggcgataaaaaacgattgggggatgagacatgaacgctcaagcagaagaaggatcc

SEQ ID NO: 92 - DNA, 362 bp, Artificial sequence
  Promoter / RNA thermometer combination 16
ggcgcctttgtggtgatctacactgatactctgttgcattattcgcctgaaaccacaatattcaggcgttttttcgctatctttgacaaaaaatatcaactttctcgatttgctctcagcccttatatcacgggaaattccggcgatttgctcgcatcaatattcatgccacatttgccatcaggggccgcctcagattctcagtatgttataatagaaaaaattaattaaggcctaattatagcacttaatcgaaataaatttatgagtacgtagagtataattagtattcttctttccaacttccttatacttatatacttatagattctaaaatcatgaaacggattctttgcggatcc

SEQ ID NO: 93 - DNA, 278 bp, Artificial sequence
  Promoter / RNA thermometer combination 17
ggcgccctggcacaggaacgttatccggacgttcagttccaccagacccgcgagcattaattcttgcctccagggcgcggtagtcgcgccctgtcaatttcccttccttattagccgcttacggaatgttcttaaaacattcacttttgcttatgttttcgctcatatcccgagcggtttcaaaattgtgatctatatttaacaaattaattaaacagcaattttgcgttatctgttaatcgagactgaaatacatgaaaaaaaccacattaggatcc

SEQ ID NO: 94 - DNA, 454 bp, Artificial sequence
  Promoter / RNA thermometer combination 18
ggcgccctggcacaggaacgttatccggacgttcagttccaccagacccgcgagcattaattcttgcctccagggcgcggtagtcgcgccctgtcaatttcccttccttattagccgcttacggaatgttcttaaaacattcacttttgcttatgttttcgctcatatcccgagcggtttcaaaattgtgatctatatttaacaaattaattaaacggtttgacgtacagaccattaaagcagtgtagtaaggcaagtcccttcaagagttatcgttgatacccctcgtagtgcacattcctttaacgcttcaaaatctgtaaagcacgccatatcgccgaaaggcacacttaattattaaaggtaatacactatgtccggtaaaatgactggtatcgtaaaatggttcaacgctgacaaaggcttcggcttcatcactcctgacgatggatcc

SEQ ID NO: 95 - DNA, 278 bp, Artificial sequence
  Promoter / RNA thermometer combination 19
ggcgccctggcacaggaacgttatccggacgttcagttccaccagacccgcgagcattaattcttgcctccagggcgcggtagtcgcgccctgtcaatttcccttccttattagccgcttacggaatgttcttaaaacattcacttttgcttatgttttcgctcatatcccgagcggtttcaaaattgtgatctatatttaacaaattaattaaacagcaattttgcgttacctgttaatcgagattgaaacacatgaaaaaaaccacattaggatcc

SEQ ID NO: 96 - DNA, 282 bp, Artificial sequence
  Promoter / RNA thermometer combination 20
ggcgccctggcacaggaacgttatccggacgttcagttccaccagacccgcgagcattaattcttgcctccagggcgcggtagtcgcgccctgtcaatttcccttccttattagccgcttacggaatgttcttaaaacattcacttttgcttatgttttcgctcatatcccgagcggtttcaaaattgtgatctatatttaacaaattaattaaattcaagggtaatcaattccttccacacatcaggagttaacattatgtctctcattctttacggatcc

SEQ ID NO: 97 - DNA, 309 bp, Artificial sequence
  Promoter / RNA thermometer combination 21
ggcgccctggcacaggaacgttatccggacgttcagttccaccagacccgcgagcattaattcttgcctccagggcgcggtagtcgcgccctgtcaatttcccttccttattagccgcttacggaatgttcttaaaacattcacttttgcttatgttttcgctcatatcccgagcggtttcaaaattgtgatctatatttaacaaattaattaaggccactttagtctgtggttactgtattaggtattgttataacaatctggatggtttttatgaataagacattactggtctcttctttaggatcc

SEQ ID NO: 98 - DNA, 356 bp, Artificial sequence
  Promoter / RNA thermometer combination 22
ggcgccctggcacaggaacgttatccggacgttcagttccaccagacccgcgagcattaattcttgcctccagggcgcggtagtcgcgccctgtcaatttcccttccttattagccgcttacggaatgttcttaaaacattcacttttgcttatgttttcgctcatatcccgagcggtttcaaaattgtgatctatatttaacaaattaattaatgtaaaaaacatcatttagcgtgactttctttcaacagctaacaattgttgttactgcctaatgtttttagggtattttaaaaaagggcgataaaaaacgattgggggatgagacatgaacgctcaagcagaagaaggatcc

SEQ ID NO: 99 - DNA, 339 bp, Artificial sequence
  Promoter / RNA thermometer combination 23
ggcgccaaaaaatattcagttacaggaaaggtcagggcagggattctacagagttctggataaaatttgtatcgcaatctcattcgctgccggaggcgaaggaaatgtaaattttgttaattcggcgtgaagaattgatcctggacagcattttgctcaaaaaatagccatactatttaattgcaacaattaattaatgtaaaaaacatcatttagcgtgactttctttcaacagctaacaattgttgttactgcctaatgtttttagggtattttaaaaaagggcgataaaaaacgattgggggatgagacatgaacgctcaagcagaagaaggatcc

SEQ ID NO: 100 - DNA, 332 bp, Artificial sequence
  Promoter / RNA thermometer combination 24
ggcgccctggcacaggaacgttatccggacgttcagttccaccagacccgcgagcattaattcttgcctccagggcgcggtagtcgcgccctgtcaatttcccttccttattagccgcttacggaatgttcttaaaacattcacttttgcttatgttttcgctcatatcccgagcggtttcaaaattgtgatctatatttaacaaattaattaatgtgttttttgtaagttctattaaatacatcagtttacagcaatgaattcaccattgtgcatcgtcaataaaaggagtgtttatgaaaaatcaatggcaacatcaatattttggatcc

SEQ ID NO: 101 - DNA, 3714 bp, Artificial sequence
  pXH plasmid 1
gttatccacagaatcaggggataacgcaggaaagaacatgtgagcaaaaggccagcaaaaggccaggaaccgtaaaaaggccgcgttgctggcgtttttccataggctccgcccccctgacgagcatcacaaaaatcgacgctcaagtcagaggtggcgaaacccgacaggactataaagataccaggcgtttccccctggaagctccctcgtgcgctctcctgttccgaccctgccgcttaccggatacctgtccgcctttctcccttcgggaagcgtggcgctttctcatagctcacgctgtaggtatctcagttcggtgtaggtcgttcgctccaagctgggctgtgtgcacgaaccccccgttcagcccgaccgctgcgccttatccggtaactatcgtcttgagtccaacccggtaagacacgacttatcgccactggcagcagccactggtaacaggattagcagagcgaggtatgtaggcggtgctacagagttcttgaagtggtggcctaactacggctacactagaagaacagtatttggtatctgcgctctgctgaagccagttaccttcggaaaaagagttggtagctcttgatccggcaaacaaaccaccgctggtagcggtggtttttttgtttgcaagcagcagattacgcgcagaaaaaaaggatctcaagaagatcctttgatcttttctacggggtctgacgctcagtggaacgaaaactcacgttaagggattttggtcatgagattatcaaaccggtgaggctatcccgttggcggttaatcacccacagcgtgaccagcttgcgctttattggccagattccaggcgagaaacctgacgtgcgagttgcatcaggctatccgccaaagctctcggagaggcagtctgggtgttcggagccagcgtggttttgcgcttaacgagagataccggaagtagttggttacccttcaccgcctgaccttgcgacagttgcagcaaacgatccacgctcgtttgacccagcaaacgaaaatcctgcttaatggtggtcaaaggcgggatgtaacagctggagtcttcggtgtcatcataacccacgacgctgatgtctgcaccaacacgcaggccggattcggtaatcgcacgcatcgcgcccagcgccatctgatcattcgccacaagcatagcggtcggaacaataccttcgttcagcatctgcatggtctgctgaaaaccgctcattgctgaccaatcgccctcgcgctcggcaatcggctgaatttgattacgcgtcaggtatttatgccaacccgccagacgcaggcgagccgacacgctgctcagcggaccggcgagcagggcgatttgctgatgacccagcgcaaccaggtgctccacgcctaatctggtgccgtcctcgtgggagaagatgatggagttaatcggagtttgatcgctaacgtccaggaacaatgccggcacgttggtgcacgcagcctccacggcgattgcgtcctggtcgtccagcgggtaattaataatcaggcctgaaacacgttgcgccaacaggttgtgcacagccgccttgcaggcctcgacaccgctgcgttcaaccatgctgacgaccacgctagcacccaactggtctgcacggctcttgatcgcggccacgatctgagacggtgcatgtaaggccaagctgctggtagcgacgccgatcagcaggctctgtttgccggccagttgttgcgctacacggttcgggatgtagttcagttccgccatcgccgcctcaactttttcacgggttttcgcgctcacgtggctcgcttgattcacaacgcgggaaactgtctgataactaacgcccgcatactcagcaacatcatatagtgttacgggtttcatattcaccaccctgaattgactctcttccgggcgctatcatgccataccgcgaaaggttttgcaccattcgatggtgtccgggatgagttccgcaagtgtgctattcaatgtttcaccgtaggcgctcactcccgatatcttgttattcctcgcagccgcgttaattaccacgacgctatccggcttgctttagaagaactcgtccagcatcaggtgaaattgcagtttgttcatgtccgggttgtcgataccatacttctgaaataagcgcttctgcaaggatgggctgaactcacccaggcaattccataggatcgccagatcctgataacgatcggcgatgcctacacggcccacgtcaatgcagccgatcagcttaccctcatcgaagatgaggttatccagggaaaaatccccatgtgtgaccacgctgtccggcgaaaacgggagcagtttatgcatttctttccacacttgttcaaccggccagccattgcgctcgtcgtcgaagtccgatgcatcaaccaggccgttgttcatacggctttgcgcttgcgccaagcggaaaacgcgatcggagttgaacgggcagttgcacaccggaatgctatgtaaacgacgcaggaacacagccagggcatcaacaatgttctcaccgctgtccgggtattcttccagaacctgaaacgcggtcttacccgggatcgcggtggtcaacagccacgcatcgtccggagtgcggataaagtgtttaatcgtcggcagaggcatgaactcggtcaaccagttcaaacgaaccatctcatccgtgacatcattagcgacagaacctttaccgtgcttaagaaacagttccggagcgtctggcttgccgtacagacgataaatggttgcgccagactgacccacgttatctcttgcccatttgtagccgtacaggtccgcgtccatattgctgttcaaacgcggacggctacatgatgtttccctttgtatgtgactcataacaccccttgtattactgtttatgtaagcagacagttttattgttcatgatgatatatttttatcttgtgcaatgtaacatcagagattttgagacacgggatcgcacaagttcactagctgaatccatccgtccgcctcatccagattgaggcgccggctgggctggctggcgcggcttgtccttgtaatacgactcactataggggaattgtgagcggataacaattccccttaattaagtatattagttaagtataagaaggagatatacatatgggaagttcacatcaccatcaccaccacggcagcggtggatccgagaacttgtattttcaaggctccaacgccctcgagtatctgcagagcggccgcatccaattgtaatcctcaatggctcggtaccaaattttcgaaaaaagacgctgaaaagcgtcttttttcgttttggtccactagtcgatgcgttcggcggatttctccccggtgctaatacgactcactataggggaattgtgagcggataacaattcccctgtagaaataattttgtttaactttaagaaggagatataccatggagatctaatgtcgacatcgagctcatcaagcttatcgttgaattcgtcgcgcttcccaggcatcaaataaaacgaaaggctcagtcgaaagactgggcctttcgttttatctgttgtttgtcggtgaacgctctctactagagtcacactggctcaccttcgggtgggcctttctgcgtttatagcggatgttagctaacgtcgtgtttaaggcgcgcc

SEQ ID NO: 102 - DNA, 3547 bp, Artificial sequence
  pXH plasmid 2
gttatccacagaatcaggggataacgcaggaaagaacatgtgagcaaaaggccagcaaaaggccaggaaccgtaaaaaggccgcgttgctggcgtttttccataggctccgcccccctgacgagcatcacaaaaatcgacgctcaagtcagaggtggcgaaacccgacaggactataaagataccaggcgtttccccctggaagctccctcgtgcgctctcctgttccgaccctgccgcttaccggatacctgtccgcctttctcccttcgggaagcgtggcgctttctcatagctcacgctgtaggtatctcagttcggtgtaggtcgttcgctccaagctgggctgtgtgcacgaaccccccgttcagcccgaccgctgcgccttatccggtaactatcgtcttgagtccaacccggtaagacacgacttatcgccactggcagcagccactggtaacaggattagcagagcgaggtatgtaggcggtgctacagagttcttgaagtggtggcctaactacggctacactagaagaacagtatttggtatctgcgctctgctgaagccagttaccttcggaaaaagagttggtagctcttgatccggcaaacaaaccaccgctggtagcggtggtttttttgtttgcaagcagcagattacgcgcagaaaaaaaggatctcaagaagatcctttgatcttttctacggggtctgacgctcagtggaacgaaaactcacgttaagggattttggtcatgagattatcaaaccggtgaggctatcccgttggcggttaatcacccacagcgtgaccagcttgcgctttattggccagattccaggcgagaaacctgacgtgcgagttgcatcaggctatccgccaaagctctcggagaggcagtctgggtgttcggagccagcgtggttttgcgcttaacgagagataccggaagtagttggttacccttcaccgcctgaccttgcgacagttgcagcaaacgatccacgctcgtttgacccagcaaacgaaaatcctgcttaatggtggtcaaaggcgggatgtaacagctggagtcttcggtgtcatcataacccacgacgctgatgtctgcaccaacacgcaggccggattcggtaatcgcacgcatcgcgcccagcgccatctgatcattcgccacaagcatagcggtcggaacaataccttcgttcagcatctgcatggtctgctgaaaaccgctcattgctgaccaatcgccctcgcgctcggcaatcggctgaatttgattacgcgtcaggtatttatgccaacccgccagacgcaggcgagccgacacgctgctcagcggaccggcgagcagggcgatttgctgatgacccagcgcaaccaggtgctccacgcctaatctggtgccgtcctcgtgggagaagatgatggagttaatcggagtttgatcgctaacgtccaggaacaatgccggcacgttggtgcacgcagcctccacggcgattgcgtcctggtcgtccagcgggtaattaataatcaggcctgaaacacgttgcgccaacaggttgtgcacagccgccttgcaggcctcgacaccgctgcgttcaaccatgctgacgaccacgctagcacccaactggtctgcacggctcttgatcgcggccacgatctgagacggtgcatgtaaggccaagctgctggtagcgacgccgatcagcaggctctgtttgccggccagttgttgcgctacacggttcgggatgtagttcagttccgccatcgccgcctcaactttttcacgggttttcgcgctcacgtggctcgcttgattcacaacgcgggaaactgtctgataactaacgcccgcatactcagcaacatcatatagtgttacgggtttcatattcaccaccctgaattgactctcttccgggcgctatcatgccataccgcgaaaggttttgcaccattcgatggtgtccgggatgagttccgcaagtgtgctattcaatgtttcaccgtaggcgctcactcccgatatcttgttattcctcgcagccgcgttaattaccacgacgctatccggcttgctttatgcaccgccctgccactcgtcgcagtattgttgcaattcattcagcatacgaccaacatggaagccgtcgcacacagcgtggtgaacctgaatcgccagcggcatcaacaccttgtcgccctgggtgtagtatttacccattgtaaataccggagcgaaaaaattatccatattggccacgttcaggtcgaagctggtgaacgaaacccacgggttcgcagaaacaaaaaacatgttttcgatgaaaccttttgggaaatacgccaggttctcaccatagcaggcaacatcttggctgtagatgtgcaaaaactggcgaaagtcatcatgatactcggaccacaggctagagaaggtttccgtttgttcgtggaacacggtgtaacacgggtgcacggaatcccaaataactaactcgccgtctttcatagccatgcggaactccggatgcgcgttcatcagacgcgccagaatatggatgaatgccggatagaacttgtgcttgttctttttgacggtcttgagaaatgcggtaatatccagctgcacagtctgattgtacgtacactgcgcgacgctttggaacgcctcaaaatgttctttacggtgccattggctgatgtccactgtagtatatcccgttatctttttttccattttagcttccttagctcctgaaaatctcgataactcaaaaaatacgcccggtagtgatcttatttcattatggtgaaagttggaacctcttatcgcacaagttcactagctgaatccatccgtccgcctcatccagattgaggcgccggctgggctggctggcgcggcttgtccttgtaatacgactcactataggggaattgtgagcggataacaattccccttaattaagtatattagttaagtataagaaggagatatacatatgggaagttcacatcaccatcaccaccacggcagcggtggatccgagaacttgtattttcaaggctccaacgccctcgagtatctgcagagcggccgcatccaattgtaatcctcaatggctcggtaccaaattttcgaaaaaagacgctgaaaagcgtcttttttcgttttggtccactagtcgatgcgttcggcggatttctccccggtgctaatacgactcactataggggaattgtgagcggataacaattcccctgtagaaataattttgtttaactttaagaaggagatataccatggagatctaatgtcgacatcgagctcatcaagcttatcgttgaattcgtcgcgcttcccaggcatcaaataaaacgaaaggctcagtcgaaagactgggcctttcgttttatctgttgtttgtcggtgaacgctctctactagagtcacactggctcaccttcgggtgggcctttctgcgtttatagcggatgttagctaacgtcgtgtttaaggcgcgcc

SEQ ID NO: 103 - DNA, 3753 bp, Artificial sequence
  pXH plasmid 3
gttatccacagaatcaggggataacgcaggaaagaacatgtgagcaaaaggccagcaaaaggccaggaaccgtaaaaaggccgcgttgctggcgtttttccataggctccgcccccctgacgagcatcacaaaaatcgacgctcaagtcagaggtggcgaaacccgacaggactataaagataccaggcgtttccccctggaagctccctcgtgcgctctcctgttccgaccctgccgcttaccggatacctgtccgcctttctcccttcgggaagcgtggcgctttctcatagctcacgctgtaggtatctcagttcggtgtaggtcgttcgctccaagctgggctgtgtgcacgaaccccccgttcagcccgaccgctgcgccttatccggtaactatcgtcttgagtccaacccggtaagacacgacttatcgccactggcagcagccactggtaacaggattagcagagcgaggtatgtaggcggtgctacagagttcttgaagtggtggcctaactacggctacactagaagaacagtatttggtatctgcgctctgctgaagccagttaccttcggaaaaagagttggtagctcttgatccggcaaacaaaccaccgctggtagcggtggtttttttgtttgcaagcagcagattacgcgcagaaaaaaaggatctcaagaagatcctttgatcttttctacggggtctgacgctcagtggaacgaaaactcacgttaagggattttggtcatgagattatcaaaccggtgaggctatcccgttggcggttaatcacccacagcgtgaccagcttgcgctttattggccagattccaggcgagaaacctgacgtgcgagttgcatcaggctatccgccaaagctctcggagaggcagtctgggtgttcggagccagcgtggttttgcgcttaacgagagataccggaagtagttggttacccttcaccgcctgaccttgcgacagttgcagcaaacgatccacgctcgtttgacccagcaaacgaaaatcctgcttaatggtggtcaaaggcgggatgtaacagctggagtcttcggtgtcatcataacccacgacgctgatgtctgcaccaacacgcaggccggattcggtaatcgcacgcatcgcgcccagcgccatctgatcattcgccacaagcatagcggtcggaacaataccttcgttcagcatctgcatggtctgctgaaaaccgctcattgctgaccaatcgccctcgcgctcggcaatcggctgaatttgattacgcgtcaggtatttatgccaacccgccagacgcaggcgagccgacacgctgctcagcggaccggcgagcagggcgatttgctgatgacccagcgcaaccaggtgctccacgcctaatctggtgccgtcctcgtgggagaagatgatggagttaatcggagtttgatcgctaacgtccaggaacaatgccggcacgttggtgcacgcagcctccacggcgattgcgtcctggtcgtccagcgggtaattaataatcaggcctgaaacacgttgcgccaacaggttgtgcacagccgccttgcaggcctcgacaccgctgcgttcaaccatgctgacgaccacgctagcacccaactggtctgcacggctcttgatcgcggccacgatctgagacggtgcatgtaaggccaagctgctggtagcgacgccgatcagcaggctctgtttgccggccagttgttgcgctacacggttcgggatgtagttcagttccgccatcgccgcctcaactttttcacgggttttcgcgctcacgtggctcgcttgattcacaacgcgggaaactgtctgataactaacgcccgcatactcagcaacatcatatagtgttacgggtttcatattcaccaccctgaattgactctcttccgggcgctatcatgccataccgcgaaaggttttgcaccattcgatggtgtccgggatgagttccgcaagtgtgctattcaatgtttcaccgtaggcgctcactcccgatatcttgttattcctcgcagccgcgttaattaccacgacgctatccggcttgctttagaagaactcgtccagcatcaggtgaaattgcagtttgttcatgtccgggttgtcgataccatacttctgaaataagcgcttctgcaaggatgggctgaactcacccaggcaattccataggatcgccagatcctgataacgatcggcgatgcctacacggcccacgtcaatgcagccgatcagcttaccctcatcgaagatgaggttatccagggaaaaatccccatgtgtgaccacgctgtccggcgaaaacgggagcagtttatgcatttctttccacacttgttcaaccggccagccattgcgctcgtcgtcgaagtccgatgcatcaaccaggccgttgttcatacggctttgcgcttgcgccaagcggaaaacgcgatcggagttgaacgggcagttgcacaccggaatgctatgtaaacgacgcaggaacacagccagggcatcaacaatgttctcaccgctgtccgggtattcttccagaacctgaaacgcggtcttacccgggatcgcggtggtcaacagccacgcatcgtccggagtgcggataaagtgtttaatcgtcggcagaggcatgaactcggtcaaccagttcaaacgaaccatctcatccgtgacatcattagcgacagaacctttaccgtgcttaagaaacagttccggagcgtctggcttgccgtacagacgataaatggttgcgccagactgacccacgttatctcttgcccatttgtagccgtacaggtccgcgtccatattgctgttcaaacgcggacggctacatgatgtttccctttgtatgtgactcataacaccccttgtattactgtttatgtaagcagacagttttattgttcatgatgatatatttttatcttgtgcaatgtaacatcagagattttgagacacgggatcgcacaagttcactagctgaatccatccgtccgcctcatccagattgaggcgccaaattttcgaaaaaagacgctgaaaagcgtcttttttcgttttggtcccgatgcgttcggcggatttctccccggtgctaatacgactcactataggggaattgtgagcggataacaattcccctgtagaaataattttgtttaactttaagaaggagatatacatatgggaagttcacatcaccatcaccaccacggcagcggtggatccgagaacttgtattttcaaggctccaacgccctcgagtatctgcagagcggccgcatccaattgtaatcctcaatggccaggcatcaaataaaacgaaaggctcagtcgaaagactgggcctttcgttttatctgttgtttgtcggtgaacgctctctactagagtcacactggctcaccttcgggtgggcctttctgcgtttataactagtggctgggctggctggcgcggcttgtccttgtaatacgactcactataggggaattgtgagcggataacaattcccctgtagaaataattttgtttaactttaataaggagatataccatggagatctaatgtcgacatcgagctcatcaagcttatcgttgaattcgtcgcgcttcctagcataaccccttggggcctctaaacgggtcttgaggggttttttggcggatgttagctaacgtcgtgtttaaggcgcgcc

SEQ ID NO: 104 - DNA, 3584 bp, Artificial sequence
  pXH plasmid 4
gttatccacagaatcaggggataacgcaggaaagaacatgtgagcaaaaggccagcaaaaggccaggaaccgtaaaaaggccgcgttgctggcgtttttccataggctccgcccccctgacgagcatcacaaaaatcgacgctcaagtcagaggtggcgaaacccgacaggactataaagataccaggcgtttccccctggaagctccctcgtgcgctctcctgttccgaccctgccgcttaccggatacctgtccgcctttctcccttcgggaagcgtggcgctttctcatagctcacgctgtaggtatctcagttcggtgtaggtcgttcgctccaagctgggctgtgtgcacgaaccccccgttcagcccgaccgctgcgccttatccggtaactatcgtcttgagtccaacccggtaagacacgacttatcgccactggcagcagccactggtaacaggattagcagagcgaggtatgtaggcggtgctacagagttcttgaagtggtggcctaactacggctacactagaagaacagtatttggtatctgcgctctgctgaagccagttaccttcggaaaaagagttggtagctcttgatccggcaaacaaaccaccgctggtagcggtggtttttttgtttgcaagcagcagattacgcgcagaaaaaaaggatctcaagaagatcctttgatcttttctacggggtctgacgctcagtggaacgaaaactcacgttaagggattttggtcatgagattatcaaaccggtgaggctatcccgttggcggttaatcacccacagcgtgaccagcttgcgctttattggccagattccaggcgagaaacctgacgtgcgagttgcatcaggctatccgccaaagctctcggagaggcagtctgggtgttcggagccagcgtggttttgcgcttaacgagagataccggaagtagttggttacccttcaccgcctgaccttgcgacagttgcagcaaacgatccacgctcgtttgacccagcaaacgaaaatcctgcttaatggtggtcaaaggcgggatgtaacagctggagtcttcggtgtcatcataacccacgacgctgatgtctgcaccaacacgcaggccggattcggtaatcgcacgcatcgcgcccagcgccatctgatcattcgccacaagcatagcggtcggaacaataccttcgttcagcatctgcatggtctgctgaaaaccgctcattgctgaccaatcgccctcgcgctcggcaatcggctgaatttgattacgcgtcaggtatttatgccaacccgccagacgcaggcgagccgacacgctgctcagcggaccggcgagcagggcgatttgctgatgacccagcgcaaccaggtgctccacgcctaatctggtgccgtcctcgtgggagaagatgatggagttaatcggagtttgatcgctaacgtccaggaacaatgccggcacgttggtgcacgcagcctccacggcgattgcgtcctggtcgtccagcgggtaattaataatcaggcctgaaacacgttgcgccaacaggttgtgcacagccgccttgcaggcctcgacaccgctgcgttcaaccatgctgacgaccacgctagcacccaactggtctgcacggctcttgatcgcggccacgatctgagacggtgcatgtaaggccaagctgctggtagcgacgccgatcagcaggctctgtttgccggccagttgttgcgctacacggttcgggatgtagttcagttccgccatcgccgcctcaactttttcacgggttttcgcgctcacgtggctcgcttgattcacaacgcgggaaactgtctgataactaacgcccgcatactcagcaacatcatatagtgttacgggtttcatattcaccaccctgaattgactctcttccgggcgctatcatgccataccgcgaaaggttttgcaccattcgatggtgtccgggatgagttccgcaagtgtgctattcaatgtttcaccgtaggcgctcactcccgatatcttgttattcctcgcagccgcgttaattaccacgacgctatccggcttgctttatgcaccgccctgccactcgtcgcagtattgttgcaattcattcagcatacgaccaacatggaagccgtcgcacacagcgtggtgaacctgaatcgccagcggcatcaacaccttgtcgccctgggtgtagtatttacccattgtaaataccggagcgaaaaaattatccatattggccacgttcaggtcgaagctggtgaacgaaacccacgggttcgcagaaacaaaaaacatgttttcgatgaaaccttttgggaaatacgccaggttctcaccatagcaggcaacatcttggctgtagatgtgcaaaaactggcgaaagtcatcatgatactcggaccacaggctagagaaggtttccgtttgttcgtggaacacggtgtaacacgggtgcacggaatcccaaataactaactcgccgtctttcatagccatgcggaactccggatgcgcgttcatcagacgcgccagaatatggatgaatgccggatagaacttgtgcttgttctttttgacggtcttgagaaatgcggtaatatccagctgcacagtctgattgtacgtacactgcgcgacgctttggaacgcctcaaaatgttctttacggtgccattggctgatgtccactgtagtatatcccgttatctttttttccattttagcttccttagctcctgaaaatctcgataactcaaaaaatacgcccggtagtgatcttatttcattatggtgaaagttggaacctcttatcgcacaagttcactagctgaatccatccgtccgcctcatccagattggcgccaaattttcgaaaaaagacgctgaaaagcgtcttttttcgttttggtcccgatgcgttcggcggatttctccccggtgctaatacgactcactataggggaattgtgagcggataacaattcccctgtagaaataattttgtttaactttaagaaggagatatacatatgggaagttcacatcaccatcaccaccacggcagcggtggatccgagaacttgtattttcaaggctccaacgccctcgagtatctgcagagcggccgcatccaattgtaatcctcaatggccaggcatcaaataaaacgaaaggctcagtcgaaagactgggcctttcgttttatctgttgtttgtcggtgaacgctctctactagagtcacactggctcaccttcgggtgggcctttctgcgtttataactagtggctgggctggctggcgcggcttgtccttgtaatacgactcactataggggaattgtgagcggataacaattcccctgtagaaataattttgtttaactttaataaggagatataccatggagatctaatgtcgacatcgagctcatcaagcttatcgttgaattcgtcgcgcttcctagcataaccccttggggcctctaaacgggtcttgaggggttttttggcggatgttagctaacgtcgtgtttaaggcgcgcc

SEQ ID NO: 105 - RNA, 29 nt, Artificial sequence
  RNA thermometer 10
ggaucccuccuucagaaggagauauaccc

SEQ ID NO: 106 - RNA, 59 nt, Artificial sequence
  RNA thermometer 11
ggauccucuccuucacuaguaaaaaaaaaaaaaaaaaaaaaaaaaaaggagauauaccc

SEQ ID NO: 107 - RNA, 29 nt, Artificial sequence
  RNA thermometer 12
ggauccucuccuuagaaggagauauaccc

SEQ ID NO: 108 - RNA, 38 nt, Artificial sequence
  RNA thermometer 13
ggaucccuccuuacuagucugcagaaggagauauaccc

SEQ ID NO: 109 - RNA, 39 nt, Artificial sequence
  RNA thermometer 14
ggauccucuccuuacuagucugcagaaggagauauaccc

SEQ ID NO: 110 - RNA, 39 nt, Artificial sequence
  RNA thermometer 15
ggaucccuccuucacuagucugcagaaggagauauaccc

SEQ ID NO: 111 - RNA, 61 nt, Artificial sequence
  RNA thermometer 16
uaaauacaucaguuuacagcaaugaauucaccauugugcaucgucaauaaaaggaguguuu